European Patent Application EP 4 458 140 A1, published November 6, 2024. Title: Tobacco Plant. Applicant: 日本たばこ産業株式会社. The sequence listing filed with the application follows.

SEQUENCE LISTING (44 sequences)

SEQ ID NO: 1 - DNA, 2361 bp, Nicotiana tabacum
  source 1..2361: mol_type = other DNA
atggaggagccaactcgattagtagaagaagcaacgattaataacatggacggacaacagaatgaagaagaaagagatccagagagcaattcactgcatcagcctcttctcaagagaaacagaacactatcatccagtccatttgccttggttggagctaaggtctcccacatcgaaagtttggattatgagatcaacgagaatgatctcttcaagcatgactggagaaggagatctagagttcaagtattacagtatgtgttcttgaaatggacactggcatttttggtcggcctgcttacaggagttacagccaccctcatcaatcttgcaatcgaaaacatggctggttacaaacttcgagctgttgtgaactatatcgaggatagaaggtaccttatgggatttgcatattttgcgggtgctaattttgtgctcactttgatagctgcccttctctgcgtgtgctttgcacctactgctgcagggcctggaattcctgaaatcaaagcttatctcaacggtgtagatactcccaatatgtatggagcaaccacactttttgtcaagatcattggaagcattgcagcagtttctgctagcttagaccttggaaaagaagggccattggttcacattggcgcttgctttgcttccttactaggtcaaggtggtccagataattaccggctcaggtggcgttggctccgttacttcaacaacgatcgggacaggcgagatcttatcacatgtgggtcatcatcaggtgtgtgtgctgctttccgttctccagtaggtggtgtcctatttgctttagaggaagtggcaacatggtggagaagtgcactcctctggagaactttcttcagcacggcagttgtggtggtgatactgagggccttcattgaatactgcaaatctggcaactgtggactttttggaagaggagggcttatcatgtttgatgtgagtggtgtcagtgttagctaccatgttgtggacatcatccctgttgtagtgattggaatcataggcggacttttgggaagcctctacaatcatgtcctccacaaaattctgaggctctacaatctgatcaacgagaagggaaaactacataaggttcttctcgctctgagtgtctcccttttcacctccatttgcatgtatggacttccttttttggccaaatgcaagccttgtgatccatcacttcccgggtcttgtcctggtactggagggacaggaaacttcaagcagttcaactgcccagacggctattacaatgatcttgctactcttctccttacaaccaacgatgatgcagtccgaaacattttctccataaacactcccggtgaattccaagttatgtctcttattatctacttcgttctgtattgcatattgggactcatcacttttgggattgctgtgccatctggtctcttccttccaatcatcctcatgggttcagcttatggtcgcttgcttgccattgccatgggatcttatacaaaaattgatccagggctgtatgcggttctcggagcagcttcccttatggctggttcaatgagaatgactgtttctctttgcgtcatatttcttgagctaacaaacaatcttctccttctgccaataacaatgctggttcttctaattgccaaaagtgtaggagactgcttcaacctaagtatttatgaaataatattggagctgaaaggtctacctttcctggatgccaacccggagccatggatgagaaatatcactgctggtgagcttgctgatgtaaagccaccagtagttacactctgtggagttgagaaggtgggacgtatcgtagaggccttgaagaacaccacatataacggattccctgtcgtcgatgaaggagtagtgccaccggtgggtctgccagttggggcaactgaattgcacggtcttgtcctaagaactcaccttcttttggttctcaagaaaaagtggttccttcatgaaagacggaggacagaggagtgggaagtgagagagaaattcacctggattgatttagctgagaggggcggtaagatcgaagatgtgttagttacaaaggatgaaatggagatgtatgtcgatttgcatcccctgactaacacaaccccttatactgtggtagaaagcttgtcagtggctaaggcaatggtgcttttcaggcaggtggggctccgccacatgctcattgtacccaaataccaagcagcaggggtatctcctgtggtgggaatcttgaccaggcaagacttgagagcccacaacattttgagtgtcttccctcatctggagaagtcaaaaagcggtaaaaaggggaactga

SEQ ID NO: 2 - protein, 786 aa, Nicotiana tabacum
MEEPTRLVEEATINNMDGQQNEEERDPESNSLHQPLLKRNRTLSSSPFALVGAKVSHIESLDYEINENDLFKHDWRRRSRVQVLQYVFLKWTLAFLVGLLTGVTATLINLAIENMAGYKLRAVVNYIEDRRYLMGFAYFAGANFVLTLIAALLCVCFAPTAAGPGIPEIKAYLNGVDTPNMYGATTLFVKIIGSIAAVSASLDLGKEGPLVHIGACFASLLGQGGPDNYRLRWRWLRYFNNDRDRRDLITCGSSSGVCAAFRSPVGGVLFALEEVATWWRSALLWRTFFSTAVVVVILRAFIEYCKSGNCGLFGRGGLIMFDVSGVSVSYHVVDIIPVVVIGIIGGLLGSLYNHVLHKILRLYNLINEKGKLHKVLLALSVSLFTSICMYGLPFLAKCKPCDPSLPGSCPGTGGTGNFKQFNCPDGYYNDLATLLLTTNDDAVRNIFSINTPGEFQVMSLIIYFVLYCILGLITFGIAVPSGLFLPIILMGSAYGRLLAIAMGSYTKIDPGLYAVLGAASLMAGSMRMTVSLCVIFLELTNNLLLLPITMLVLLIAKSVGDCFNLSIYEIILELKGLPFLDANPEPWMRNITAGELADVKPPVVTLCGVEKVGRIVEALKNTTYNGFPVVDEGVVPPVGLPVGATELHGLVLRTHLLLVLKKKWFLHERRRTEEWEVREKFTWIDLAERGGKIEDVLVTKDEMEMYVDLHPLTNTTPYTVVESLSVAKAMVLFRQVGLRHMLIVPKYQAAGVSPVVGILTRQDLRAHNILSVFPHLEKSKSGKKGN

SEQ ID NO: 3 - DNA, 2361 bp, Nicotiana tabacum
  source 1..2361: mol_type = other DNA
atggaggagccaactcgattagtagaagaagcaacgattaataacatggacagacaacagaatgaagaagaaagagatccagagagcaattcactgcatcagcctctcctcaagagaaacagaacactatcatccagtccatttgccttggttggagctaaggtctcccatattgaaagtttagactatgagatcaacgagaatgatctcttcaagcatgactggagaagaagatccagagttcaagtattacagtatgtattcttgaaatggacactggcatttttggtcgggcttcttacaggagtgacagcctcccttatcaatcttgcaatcgaaaacattgctggctacaaacttagagctgttgtgaactatatcgaggatagaaggtaccttgtgggatttgcatattttgcgggtgctaattttgtgctcactttgatagctgcccttctctgcgtgtgttttgcgcctactgctgcagggcctggaattcctgaaatcaaagcttatctcaacggtgtagatactcccaacatgtacggagcaaccacactttttgtcaagatcattggaagcattgcagcagtttctgctagcttagaccttggaaaagaagggccgttggttcacattggcgcttgttttgcttccttactaggtcaaggtggtccagataattaccggctcaaatggcgctggctccgttacttcaacaacgatcgggacaggcgagatctcatcacatgtgggtcatcatcaggtgtgtgtgctgctttccgttctccagtaggtggtgtcctatttgctttagaggaagtggcaacatggtggagaagtgcactcctctggagaactttcttcagcacggcagttgtggtggtgatactgagggccttcatagaatactgcaaatctggctactgtggactttttggaagaggagggcttatcatgtttgatgtgagtggtgtcagtgttagctaccatgttgtggacatcatccctgttgttgtgattggaatcataggcggacttttgggaagcctctacaattgtgtcctccacaaagttctgaggctctacaatctcatcaacgagaagggaaaactacataaggttcttctcgctctgagcgtctcccttttcacctccatttgcatgtatggacttccttttttggccaaatgcaagccttgtgattcatcacttcaagggtcttgtcctggcactggaggtacaggaaacttcaagcagttcaactgccctgacggctattacaatgatctcgctactcttctccttacaaccaacgatgatgcagtccgaaacattttctccataaacactcccggtgaattccatgttacgtctcttattatctacttcgttctgtattgtatcttgggactcatcacttttgggattgctgtgccatctggtctcttccttccaatcatcctcatgggttcagcttatggtcgcttgcttgccattgccatgggatcttatacaaaaattgatccagggctgtatgccgttctgggagcagcttcccttatggctggttcaatgagaatgactgtttctctttgcgtcatatttcttgagctaacaaacaatcttctccttctgccaataacaatgctggttcttctaattgccaaaagtgtaggagactgctttaacctaagtatttatgaaataatattggaactgaaaggtctacctttcctggatgccaacccggagccatggatgagaaatatcactgctggtgagcttgctgatgtaaagccaccagtagttacactttgtggagttgagaaggtgggacgtatcgtcgaggtcttgaagaacaccacatataacggattccctgtcgtcgatgaaggagtggtgccaccggtgggtctgccagttggggcaactgaattgcacggtcttgtcctaagaactcaccttcttttggttctcaagaaaaagtggttccttaatgaaagacgaaggacagaggagtgggaagtgagagagaaattcacctggattgatttagctgagaggggcggtaagatcgaagatgtggtagttacgaaggatgaaatggagatgtatgtcgatttgcatcccctgactaacacaaccccttatactgtggtagaaagcttgtcagtggctaaggcaatggtgcttttcaggcaggtggggctccgccacatgctcattgtacccaaataccaagcagcaggggtatctccggtggtgggaatcttgaccaggcaagacttgagagcccacaacattttgagtgtcttccctcatctggagaagtcaaaaagcggtaaaaaggggaactga

SEQ ID NO: 4 - protein, 786 aa, Nicotiana tabacum
MEEPTRLVEEATINNMDRQQNEEERDPESNSLHQPLLKRNRTLSSSPFALVGAKVSHIESLDYEINENDLFKHDWRRRSRVQVLQYVFLKWTLAFLVGLLTGVTASLINLAIENIAGYKLRAVVNYIEDRRYLVGFAYFAGANFVLTLIAALLCVCFAPTAAGPGIPEIKAYLNGVDTPNMYGATTLFVKIIGSIAAVSASLDLGKEGPLVHIGACFASLLGQGGPDNYRLKWRWLRYFNNDRDRRDLITCGSSSGVCAAFRSPVGGVLFALEEVATWWRSALLWRTFFSTAVVVVILRAFIEYCKSGYCGLFGRGGLIMFDVSGVSVSYHVVDIIPVVVIGIIGGLLGSLYNCVLHKVLRLYNLINEKGKLHKVLLALSVSLFTSICMYGLPFLAKCKPCDSSLQGSCPGTGGTGNFKQFNCPDGYYNDLATLLLTTNDDAVRNIFSINTPGEFHVTSLIIYFVLYCILGLITFGIAVPSGLFLPIILMGSAYGRLLAIAMGSYTKIDPGLYAVLGAASLMAGSMRMTVSLCVIFLELTNNLLLLPITMLVLLIAKSVGDCFNLSIYEIILELKGLPFLDANPEPWMRNITAGELADVKPPVVTLCGVEKVGRIVEVLKNTTYNGFPVVDEGVVPPVGLPVGATELHGLVLRTHLLLVLKKKWFLNERRRTEEWEVREKFTWIDLAERGGKIEDVVVTKDEMEMYVDLHPLTNTTPYTVVESLSVAKAMVLFRQVGLRHMLIVPKYQAAGVSPVVGILTRQDLRAHNILSVFPHLEKSKSGKKGN

SEQ ID NO: 5 - DNA, 2361 bp, Nicotiana tabacum; identical to SEQ ID NO: 1
  source 1..2361: mol_type = other DNA

SEQ ID NO: 6 - protein, 786 aa, Nicotiana tabacum; identical to SEQ ID NO: 2

SEQ ID NO: 7 - DNA, 2721 bp, Nicotiana tabacum
  source 1..2721: mol_type = other DNA
atgattagcggccaaaacaccgtgctgcaccatcctcctaattcgctcttcaattccttatctcctcgccatatctgtgtatctttctgtaacgacaaagctttaaaaaagtcagtcacgcactccgcccctcggtttgctcgtctgttaaacaatgaatcacgaaagttgttgggtcgtcatccaaattgctggccttgggctcgacgaccatctcttcctccgggacgttcctgtgacggaaacattgaaaaagaacaagatatgtgcgacagcagcaaagacgatagtgatagtgatagtggtatccagataggatctctgctcgaggaagttatcccacaaggcaataataccgctataatctcggcttgctttgttggcctcttcaccggtatcagtgtcgtgcttttcaacgctgcggttcatgaaatacgtgatctttgttgggatggaattccatatcgagctgcctcagaggagcccattggagtacattggcaacgtgtaatcttagtaccagcttgtggcggtttggtagtcagctttttgaatgccttccgagccactctggaggtttcaactgaagaaagttggacatcatctgttaaatctgtgttggggccagttttgaagacaatggccgcttgtgtcacattaggaactgggaattccttaggaccagaaggccctagtgttgaaattggtacatctgttgccaagggagttggagctctgcttgataaaggtggtcgtagaaagctgtcactcaaggctgctggatcagctgctggaatcgcttctggatttaatgctgctgtcgggggctgtttctttgctgtggaatctgtgttatggccatcacctgcagagtcctccttgtacttgacaaatacgacttcaatggttattctcagtgctgttatagcttctgtagtctcagaaattggtcttggctctgaacctgcatttgcagttccaggatatgatttccgtacacctactgagctgccgctttatcttctgctgggcatcttttgtggcttagtttcagtggcattatcaagttgtacatcatttatgctgcaaatagtggaaaatattcaaatgaccagcggcatgccaaaagcagcttttcctgtcctgggcggtcttctggttgggctggtagctttagcatatcctgaaatcctttaccagggttttgagaatgttaatattctgctagaatctcgcccactagtgaaaggcctctccgctgatctgttgctccagcttgtagctgtcaaaatagtaacaacttcattatgccgagcctctggattggttggaggctactatgcgccatctctattcatcggtgctgctactggaactgcatatgggaaaattgttagctacattatctctcatgctgatccaatctttcatctttccatcttggaagttgcatccccacaagcttatggcctggttggcatggctgctactcttgctggtgtctgtcaggtgcctctcactgctgttttgcttctctttgaactgacacagaattatcggatagttctgcccctcttgggagctgtggggttgtcttcttgggttacatctggacaaacaaggaaaagtgtagtgaaggatagagaaagactaaaagatgcaagagcccacatgatgcagcgacaaggaacttctttctccaacatttctagtttaacttattcttcaggtgtgaaaccttcacagaaagagagtaacctatgcaaacttgagagttccctctgtctttatgaatctgatgatgaagaaaatgatttggcaaggacaattctagtttcacaggcaatgagaacacgatatgtgacagttctaatgagcaccttgctaacggagaccatatccctcatgctagctgagaagcaatcttgtgcaataatagttgatgaaaataattttctcattggtctgctgacacttagtgatatccagaattacagcaagttgccaagagcagagggcaatttccaggagatcaacttgattggcacagagcttatgaaaagagtttctcaggcggaccggcaagttatagatttgcgcaccgaggctgataactggaaggaacaattcgaaggtcttcaattggaaaaagaggttccggcggaagagaagaatgctttggaacaacagatgagagtgattgcctctgaattagcagttgaaaaagcttcctcgagccaggttggaaaggataagtatatacttgaatcctcctttgctgaacaactttccaaggcaactgaagaaataaggagtttgaaggaactccttaatcaaaaagaggtttatgcgagagaattggttcaaacacttactcaagttcaggaagatctccgtgcctctacttataagattcagttcttggaaagttctctcgcttctttgaagacagcttacgatgcctctgaagcagaaaaagaagagttgagagctgagatttaccagtgggagaaggattatgagattctcgaggataatctatcgttggatgtaagttgggctttcttaaacactcgtctcgagactctagttgaagccaaccatgagggttttgaccttaatgctgagattgctaaggctaaagaagcaattgataaaactcagcaacgtcaaatcttttcctcacctgaagacgaaggtcccgaaggtgatggagattga

SEQ ID NO: 8 - protein, 906 aa, Nicotiana tabacum
MISGQNTVLHHPPNSLFNSLSPRHICVSFCNDKALKKSVTHSAPRFARLLNNESRKLLGRHPNCWPWARRPSLPPGRSCDGNIEKEQDMCDSSKDDSDSDSGIQIGSLLEEVIPQGNNTAIISACFVGLFTGISVVLFNAAVHEIRDLCWDGIPYRAASEEPIGVHWQRVILVPACGGLVVSFLNAFRATLEVSTEESWTSSVKSVLGPVLKTMAACVTLGTGNSLGPEGPSVEIGTSVAKGVGALLDKGGRRKLSLKAAGSAAGIASGFNAAVGGCFFAVESVLWPSPAESSLYLTNTTSMVILSAVIASVVSEIGLGSEPAFAVPGYDFRTPTELPLYLLLGIFCGLVSVALSSCTSFMLQIVENIQMTSGMPKAAFPVLGGLLVGLVALAYPEILYQGFENVNILLESRPLVKGLSADLLLQLVAVKIVTTSLCRASGLVGGYYAPSLFIGAATGTAYGKIVSYIISHADPIFHLSILEVASPQAYGLVGMAATLAGVCQVPLTAVLLLFELTQNYRIVLPLLGAVGLSSWVTSGQTRKSVVKDRERLKDARAHMMQRQGTSFSNISSLTYSSGVKPSQKESNLCKLESSLCLYESDDEENDLARTILVSQAMRTRYVTVLMSTLLTETISLMLAEKQSCAIIVDENNFLIGLLTLSDIQNYSKLPRAEGNFQEINLIGTELMKRVSQADRQVIDLRTEADNWKEQFEGLQLEKEVPAEEKNALEQQMRVIASELAVEKASSSQVGKDKYILESSFAEQLSKATEEIRSLKELLNQKEVYARELVQTLTQVQEDLRASTYKIQFLESSLASLKTAYDASEAEKEELRAEIYQWEKDYEILEDNLSLDVSWAFLNTRLETLVEANHEGFDLNAEIAKAKEAIDKTQQRQIFSSPEDEGPEGDGD

SEQ ID NO: 9 - DNA, 20 bp, synthetic construct
  misc_feature 1..20: note = 220S-F primer
  source 1..20: mol_type = other DNA
attaccggctcaggtggcgt

SEQ ID NO: 10 - DNA, 20 bp, synthetic construct
  misc_feature 1..20: note = 220S-R primer
  source 1..20: mol_type = other DNA
tgccagatttgcagtattca

SEQ ID NO: 11 - DNA, 20 bp, synthetic construct
  misc_feature 1..20: note = 222T-F primer
  source 1..20: mol_type = other DNA
cttaccaactcctttttccc

SEQ ID NO: 12 - DNA, 19 bp, synthetic construct
  misc_feature 1..19: note = 222T-R primer
  source 1..19: mol_type = other DNA
tgtgataaaaagaccatgt

SEQ ID NO: 13 - DNA, 20 bp, synthetic construct
  misc_feature 1..20: note = 223T-F primer
  source 1..20: mol_type = other DNA
ataattaccggctcaaatgg

SEQ ID NO: 14 - DNA, 19 bp, synthetic construct
  misc_feature 1..19: note = 223T-R primer
  source 1..19: mol_type = other DNA
tgtgataaaaagaccatgt

SEQ ID NO: 15 - DNA, 21 bp, synthetic construct
  misc_feature 1..21: note = S/T_FW1 primer
  source 1..21: mol_type = other DNA
ttggtctgacgaagttgtacg

SEQ ID NO: 16 - DNA, 20 bp, synthetic construct
  misc_feature 1..20: note = S_RT_F1 primer
  source 1..20: mol_type = other DNA
atcgcttctggatttaatgc

SEQ ID NO: 17 - DNA, 20 bp, synthetic construct
  misc_feature 1..20: note = S_RT_F2 primer
  source 1..20: mol_type = other DNA
atatggcctggttggcatgg

SEQ ID NO: 18 - DNA, 20 bp, synthetic construct
  misc_feature 1..20: note = S/T_RT_R1 primer
  source 1..20: mol_type = other DNA
ttcatgaaccgcagcgttga

SEQ ID NO: 19 - DNA, 20 bp, synthetic construct
  misc_feature 1..20: note = S_RT_R2 primer
  source 1..20: mol_type = other DNA
gcattaaatccagaagcgat

SEQ ID NO: 20 - DNA, 20 bp, synthetic construct
  misc_feature 1..20: note = S_RT_R3 primer
  source 1..20: mol_type = other DNA
agcctttccttcgtggagaa

SEQ ID NO: 21 - DNA, 20 bp, synthetic construct
  misc_feature 1..20: note = S_RT_R4 primer
  source 1..20: mol_type = other DNA
aaccgcagtgagaggcacct

SEQ ID NO: 22 - DNA, 20 bp, synthetic construct
  misc_feature 1..20: note = T_RT_F1 primer
  source 1..20: mol_type = other DNA
tcaacgctgcggttcatgaa

SEQ ID NO: 23 - DNA, 20 bp, synthetic construct
  misc_feature 1..20: note = T_RT_F2 primer
  source 1..20: mol_type = other DNA
gtacacctactgagctgccg

SEQ ID NO: 24 - DNA, 19 bp, synthetic construct
  misc_feature 1..19: note = T_RT_F3 primer
  source 1..19: mol_type = other DNA
ttatggcctggttggcatg

SEQ ID NO: 25 - DNA, 21 bp, synthetic construct
  misc_feature 1..21: note = T_RT_F4 primer
  source 1..21: mol_type = other DNA
ctcattggtctgctgacactt

SEQ ID NO: 26 - DNA, 20 bp, synthetic construct
  misc_feature 1..20: note = T_RT_R2 primer
  source 1..20: mol_type = other DNA
cggcagctcagtaggtgtac

SEQ ID NO: 27 - DNA, 22 bp, synthetic construct
  misc_feature 1..22: note = T_RT_R3 primer
  source 1..22: mol_type = other DNA
gaagaagaggcttgaacatcag

SEQ ID NO: 28 - DNA, 20 bp, synthetic construct
  misc_feature 1..20: note = CLCa_qRT-PCR_F3 primer
  source 1..20: mol_type = other DNA
catggacggacaacagaatg

SEQ ID NO: 29 - DNA, 20 bp, synthetic construct
  misc_feature 1..20: note = CLCa_qRT-PCR_R3 primer
  source 1..20: mol_type = other DNA
gggagaccttagctccaacc

SEQ ID NO: 30 - DNA, 20 bp, synthetic construct
  misc_feature 1..20: note = CLCa_qRT-PCR_F7 primer
  source 1..20: mol_type = other DNA
attggttcacattggcgctt

SEQ ID NO: 31 - DNA, 20 bp, synthetic construct
  misc_feature 1..20: note = CLCa_qRT-PCR_R7 primer
  source 1..20: mol_type = other DNA
ataagatctcgcctgtcccg

SEQ ID NO: 32 - DNA, 20 bp, synthetic construct
  misc_feature 1..20: note = CLCa_qRT-PCR_F4 primer
  source 1..20: mol_type = other DNA
cttgctttgttggcctcttc

SEQ ID NO: 33 - DNA, 20 bp, synthetic construct
  misc_feature 1..20: note = CLCa_qRT-PCR_R4 primer
  source 1..20: mol_type = other DNA
tgtactccaatgggctcctc

SEQ ID NO: 34 - DNA, 20 bp, synthetic construct
  misc_feature 1..20: note = CLCa_qRT-PCR_F6 primer
  source 1..20: mol_type = other DNA
acgaaagttgttgggtcgtc

SEQ ID NO: 35 - DNA, 20 bp, synthetic construct
  misc_feature 1..20: note = CLCa_qRT-PCR_R6 primer
  source 1..20: mol_type = other DNA
tatcgtctttgctgctgtcg

SEQ ID NO: 36 - DNA, 20 bp, synthetic construct
  misc_feature 1..20: note = ribosomal protein L25_qRT_F primer
  source 1..20: mol_type = other DNA
cccctcaccacagagtctgc

SEQ ID NO: 37 - DNA, 24 bp, synthetic construct
  misc_feature 1..24: note = ribosomal protein L25_qRT_R primer
  source 1..24: mol_type = other DNA
aagggtgttgttgtcctcaatctt

SEQ ID NO: 38 - DNA, 21 bp, synthetic construct
  misc_feature 1..21: note = CLCa_S_F1 primer
  source 1..21: mol_type = other DNA
catgactggagaaggagatct

SEQ ID NO: 39 - DNA, 22 bp, synthetic construct
  misc_feature 1..22: note = CLCa_S_R1 primer
  source 1..22: mol_type = other DNA
aagtgtggttgctccatacata

SEQ ID NO: 40 - DNA, 20 bp, synthetic construct
  misc_feature 1..20: note = CLCa_220S_R primer
  source 1..20: mol_type = other DNA
tgccagatttgcagtattca

SEQ ID NO: 41 - DNA, 2715 bp, Nicotiana tabacum
  source 1..2715: mol_type = other DNA
atggcggcatctgtcgaaaacaggcagttcagtcacatagaagccggtttatcccggtctttcaagcctcggtctgattccccggttcgtggctgcaacttccctccgcccaacagtactaatttccaaaagaaaccaaattccaccattttccttgattactcgtcgagtgaagacgacgatgatgatgacgaaaaaaatgagtaccttcaaatgatcaaaaaagggaattcagaattagagccatctgttcatgacagcagggacgaaggtaccgctgataactggattgaacgcaacttttccttgattcgtctcaccggaaagcatccatttaactccgaaccgccgttgaaccgtctcatgcaccacggttttatcacaccggtcccacttcattacgttcgtaaccatggaccggttcccaagggcacatgggatgactggaccgtggaagtcacgggactagtgaaacgtcctatgaaattcacaatggaccagttggttaacgaattcccttccagagaattgcccgttacgcttgtgtgtgctggcaaccgaaggaaagaacagaacatggttaaacaaaccattggtttcaactggggtgccgctgccgtttcaacaactgtatggcgcggggtacccctacgcgctttgttaaaacggtgcggtgtttttagcaagaataaaggggcgcttaatgtttgcttcgaaggagctgatgtcttgcccggaggcggtggttcaaagtatggaaccagcattaagaaggaatttgcaatggatccagcacgagatatcataatagcttacatgcagaacggagaaaaattggcacccgaccacgggtttccagtacgaatgataattccaggattcattggaggaagaatggtgaaatggataaagaggattatagtcaccacccaagaatcagacagctattatcatttcaaggacaatagagttcttcctccccatgttgatgctgaacttgcaaatactgaagcatggtggtacaagccagagtacatcatcaatgagctcaatattaactctgtcattacgacgccgtgtcatgaagaaattttgcctattaacgcctggacgactcagcgaccttacacgttgaggggctattcttattctggcggagggaaaaaagtaacgcgagtagaagtgaccttggatggaggagaaacatggcaagtttgcacactagatcacccagagaagcccaccaaatatggcaagtactggtgttggtgcttttggtcactcgaggttgaggtgttagacttgctcagtgccaaagaaattgctgttcgagcttgggatgagaccctcaatactcaacctgagaagcttatttggaatgtcatgggaatgatgaacaattgctggttccgagtaaagatgaatgtgtgcaagcctcacaagggagagattggaatagtgtttgaacacccgactcaacctggaaaccaatcaggtggatggatggcaaaggagaggcatttggagatatcagcagaggcacctccaacactaaagaagagtatctcaactccattcatgaacacagcttccaagatgtactccatgtcggaggtgaggaaacacagctctgctgactctgcttggatcatagtccatggtcatatctatgacgccacgcgtttcttgaaagatcaccccggtggttctgacagcattctcatcaatgctggcactgattgcactgaggaatttgatgcaattcattctgataaggctaagaagctattggaggaattcaggattggtgaactcataactactggttacacctctgactctcctggcaactccgtccatggatcttcttccttcagcagctttctagcacctattaaggaacttgttccagcgcagaggagtgtggccctcattccaagagagaaaatcccatgcaaactcatcgacaaacaatccatctcccctgatgttaggaaatttcgatttgcattgccctctgaggatcaagtcttgggcttgcctgttggtaaacacatcttcctctgtgccgttattgacgataagctctgcatgcgcgcctacacgcctactagcacgatcgatgaggtggggtacttcgagttggttgtcaagatatacttcaaaggaattcaccctaaattccccaatggggggcaaatgtcacaataccttgattctctccaattagggtcatttctcgacgtgaaaggtccattaggtcacattgaataccaaggaaagggcaatttcttagttcatggcaaacaaaagtttgccaagaagttggccatgatagcaggtggaacagggataactccagtttatcaagtcatgcaggcaattctgaaagatccagaagatgacacagaaatgtatgtggtctatgctaatagaacagaggatgatattttacttaaggaagagcttgattcatgggctgagaaaattccagaaagggttaaagtttggtatgtggttcaagattctattaaagaaggatggaagtacagccttggttttatttcagaagccattttgagagaacatatccctgagccatctcacacaacactggctttggcttgtggaccacctcctatgattcaatttgctgttaatccaaacttggagaagatgggctatgacattaaggattccttattggtgttctaa

SEQ ID NO: 42 - protein, 904 aa, Nicotiana tabacum
MAASVENRQFSHIEAGLSRSFKPRSDSPVRGCNFPPPNSTNFQKKPNSTIFLDYSSSEDDDDDDEKNEYLQMIKKGNSELEPSVHDSRDEGTADNWIERNFSLIRLTGKHPFNSEPPLNRLMHHGFITPVPLHYVRNHGPVPKGTWDDWTVEVTGLVKRPMKFTMDQLVNEFPSRELPVTLVCAGNRRKEQNMVKQTIGFNWGAAAVSTTVWRGVPLRALLKRCGVFSKNKGALNVCFEGADVLPGGGGSKYGTSIKKEFAMDPARDIIIAYMQNGEKLAPDHGFPVRMIIPGFIGGRMVKWIKRIIVTTQESDSYYHFKDNRVLPPHVDAELANTEAWWYKPEYIINELNINSVITTPCHEEILPINAWTTQRPYTLRGYSYSGGGKKVTRVEVTLDGGETWQVCTLDHPEKPTKYGKYWCWCFWSLEVEVLDLLSAKEIAVRAWDETLNTQPEKLIWNVMGMMNNCWFRVKMNVCKPHKGEIGIVFEHPTQPGNQSGGWMAKERHLEISAEAPPTLKKSISTPFMNTASKMYSMSEVRKHSSADSAWIIVHGHIYDATRFLKDHPGGSDSILINAGTDCTEEFDAIHSDKAKKLLEEFRIGELITTGYTSDSPGNSVHGSSSFSSFLAPIKELVPAQRSVALIPREKIPCKLIDKQSISPDVRKFRFALPSEDQVLGLPVGKHIFLCAVIDDKLCMRAYTPTSTIDEVGYFELVVKIYFKGIHPKFPNGGQMSQYLDSLQLGSFLDVKGPLGHIEYQGKGNFLVHGKQKFAKKLAMIAGGTGITPVYQVMQAILKDPEDDTEMYVVYANRTEDDILLKEELDSWAEKIPERVKVWYVVQDSIKEGWKYSLGFISEAILREHIPEPSHTTLALACGPPPMIQFAVNPNLEKMGYDIKDSLLVF

SEQ ID NO: 43 - DNA, 2715 bp, Nicotiana tabacum
  source 1..2715: mol_type = other DNA
atggcggcatctgtcgaaaacaggcagttcagtcacctagaagccggtttatcccggtctttcaagccccggtctgattccccggttcgtggctgcaacttcccttcgcccaacagtactaatttccaaaagaaaccaaattccaccatttaccttgattactcgtcgagtgaagacgacgatgatgatgacgaaaaaaatgagtaccttcaaatgattaaaaaagggaattcagagttagagccatctgttcatgacactagggacgaaggtaccgctgataattggattgaacgcaacttttccatgattcgtctcaccggaaagcatccatttaactccgaaccaccgttgaaccggctcatgcaccacggctttatcacaccggtcccacttcattacgttcgtaaccatggaccggttcccaagggcacgtgggatgactggaccgtggaagtcacgggactagtgaagcgtcctatgaaattcacaatggaccagttggttaacgaattcccttgtagagaattgcccgttacgcttgtttgtgctggcaatcgaaggaaagaacagaacatggttaaacaaaccattggtttcaactggggcgccgctgccgtttcaacaacgatatggcgcggggtacccctccgcgctttgctaaaacggtgcggtgtttttagcaagaataaaggggcgcttaatgtttgcttcgaaggagctgatgtgttgcccggaggtggtggttcaaagtatggaaccagcattaagaaggaatttgcaatggatccagcacgagatatcatcgtagcctacatgcagaacggagaaaaattggcacccgaccacgggtttccagtacgaatgataattccaggattcattggaggaagaatggtgaaatggataaagaggattatagtcaccacccaagaatcagacagctattatcatttcaaggacaatagagttcttcctccccatgttgatgctgaacttgcaaataccgaagcatggtggtacaagccagagtatatcatcaatgagcttaatattaactctgtcattacgacgccgtgtcatgaagaaattttgccaattaacgcctggacgactcagcgaccttacacgttgaggggctattcttattctggcggagggaaaaaagtaacgcgagtagaagtgacgttggatggaggagaaacatggcaagttagcacactagatcacccagagaagcccaccaaatatggcaagtactggtgttggtgcttttggtcactcgaggttgaggtgttagacttgctcagtgctaaagaaattgctgttcgagcttgggatgagaccctcaatactcaacccgagaagcttatttggaacgtcatgggaatgatgaataattgctggttccgagtaaagatgaatgtgtgcaagcctcacaagggagagattggaatagtgtttgagcatccgactcaacctggaaaccaatcaggtggatggatggcgaaggagagacatttggagatatcagcagaggcacctcaaacactaaagaagagtatctcaactccattcatgaacacagcttccaagatgtactccatgtccgaggtcaggaaacacagctctgctgactctgcttggatcatagtccatggtcatatctatgacgccacgcgtttcttgaaagatcaccctggtgggactgacagcattctcatcaatgctggcactgattgcactgaggaatttgatgcaattcattctgataaggctaagaagctcttggaggatttcaggattggtgaactcataactactggttacacctctgactctcctggcaactccgtgcacggatcttcttccttcagcagctttctagcacctattaaggaacttgttccagcgcagaggagtgtggccctaattccaagagagaaaatcccatgcaaactcatcgacaagcaatccatctcccatgatgttaggaaatttcgatttgcattgccctctgaggatcaagtcttgggcttgcctgttggaaaacatatcttcctctgtgccgttattgacgataagctctgcatgcgcgcttacacgcctactagcacgatcgatgaggtggggtacttcgagttggttgtcaagatatacttcaaaggaattcaccctaaattccccaatggagggcaaatgtcacagtatcttgattctatgccgttagggtcatttctcgacgtgaaaggtccattaggtcacattgaataccaaggaaagggaaatttcttagttcatggcaaacagaagtttgccaagaagttggccatgatagcaggtggaacaggaataactccagtgtatcaagtcatgcaggcaattctgaaagatccagaagatgacacagaaatgtatgtggtgtatgctaacagaacagaggatgatattttacttaaggaagagcttgattcatgggctgagaaaattccagagagggttaaagtttggtatgtggttcaggattctattaaagaaggatggaagtacagcattggttttattacagaagccattttgagagaacatatccctgagccatctcacacaacactggctttggcttgtggaccacctcctatgattcaatttgctgttaatccaaacttggagaagatgggctatgacattaaggattccttattggtgttctaa

SEQ ID NO: 44 - protein, 904 aa, Nicotiana tabacum
MAASVENRQFSHLEAGLSRSFKPRSDSPVRGCNFPSPNSTNFQKKPNSTIYLDYSSSEDDDDDDEKNEYLQMIKKGNSELEPSVHDTRDEGTADNWIERNFSMIRLTGKHPFNSEPPLNRLMHHGFITPVPLHYVRNHGPVPKGTWDDWTVEVTGLVKRPMKFTMDQLVNEFPCRELPVTLVCAGNRRKEQNMVKQTIGFNWGAAAVSTTIWRGVPLRALLKRCGVFSKNKGALNVCFEGADVLPGGGGSKYGTSIKKEFAMDPARDIIVAYMQNGEKLAPDHGFPVRMIIPGFIGGRMVKWIKRIIVTTQESDSYYHFKDNRVLPPHVDAELANTEAWWYKPEYIINELNINSVITTPCHEEILPINAWTTQRPYTLRGYSYSGGGKKVTRVEVTLDGGETWQVSTLDHPEKPTKYGKYWCWCFWSLEVEVLDLLSAKEIAVRAWDETLNTQPEKLIWNVMGMMNNCWFRVKMNVCKPHKGEIGIVFEHPTQPGNQSGGWMAKERHLEISAEAPQTLKKSISTPFMNTASKMYSMSEVRKHSSADSAWIIVHGHIYDATRFLKDHPGGTDSILINAGTDCTEEFDAIHSDKAKKLLEDFRIGELITTGYTSDSPGNSVHGSSSFSSFLAPIKELVPAQRSVALIPREKIPCKLIDKQSISHDVRKFRFALPSEDQVLGLPVGKHIFLCAVIDDKLCMRAYTPTSTIDEVGYFELVVKIYFKGIHPKFPNGGQMSQYLDSMPLGSFLDVKGPLGHIEYQGKGNFLVHGKQKFAKKLAMIAGGTGITPVYQVMQAILKDPEDDTEMYVVYANRTEDDILLKEELDSWAEKIPERVKVWYVVQDSIKEGWKYSIGFITEAILREHIPEPSHTTLALACGPPPMIQFAVNPNLEKMGYDIKDSLLVF